European Patent Application EP 4 707 304 A1, published March 11, 2026. Title: hCLDN6的抗原结合蛋白和其用途. Applicant: 泰诚思(上海)生物医药有限公司. Application CN. The sequence listing filed with the application follows.

SEQUENCE LISTING (171 sequences)

SEQ ID NO: 1 - protein, 119 aa, synthetic construct
EVKLVESGGGLVKPGGSLKLSCAASGFTFNSYTMSWVRQTPAKRLEWVVTISSGGGRTYYPDSVKGRFTISRDNARNTLYLQMSSLRSEDTAMYYCIRGDYRYDGFAYWGQGTLVTVST

SEQ ID NO: 2 - protein, 5 aa, Mus musculus
SYTMS

SEQ ID NO: 3 - protein, 17 aa, Mus musculus
TISSGGGRTYYPDSVKG

SEQ ID NO: 4 - protein, 10 aa, Mus musculus
GDYRYDGFAY

SEQ ID NO: 5 - protein, 107 aa, synthetic construct
DIQMTQSPASLSASVGETVTITCRASENIDSYLAWYQQKQGKSPQLLVYASTLLVDGVPSRFSGSRSGTQFSLKINSLQSEDVARYYCQHYYSIPYTFGSGTKLEIK

SEQ ID NO: 6 - protein, 11 aa, Mus musculus
RASENIDSYLA

SEQ ID NO: 7 - protein, 7 aa, Mus musculus
ASTLLVD

SEQ ID NO: 8 - protein, 9 aa, Mus musculus
QHYYSIPYT

SEQ ID NO: 9 - protein, 330 aa, Homo sapiens
ASTKGPSVFPLAPSSKSTSGGTAALGCLVKDYFPEPVTVSWNSGALTSGVHTFPAVLQSSGLYSLSSVVTVPSSSLGTQTYICNVNHKPSNTKVDKKVEPKSCDKTHTCPPCPAPELLGGPSVFLFPPKPKDTLMISRTPEVTCVVVDVSHEDPEVKFNWYVDGVEVHNAKTKPREEQYNSTYRVVSVLTVLHQDWLNGKEYKCKVSNKALPAPIEKTISKAKGQPREPQVYTLPPSREEMTKNQVSLTCLVKGFYPSDIAVEWESNGQPENNYKTTPPVLDSDGSFFLYSKLTVDKSRWQQGNVFSCSVMHEALHNHYTQKSLSLSPGK

SEQ ID NO: 10 - protein, 107 aa, Homo sapiens [sequence omitted]

SEQ ID NO: 11 - protein, 119 aa, synthetic construct
EVQLVESGGGLVKPGGSLRLSCAASGFTFNSYTMNWVRQAPGKGLEWVVTISSGGGRTYYPDSVKGRFTISRDNAKNSLYLQMNSLRAEDTAVYYCIRGDYRYDGFAYWGQGTLVTVSS

SEQ ID NO: 12 - protein, 119 aa, synthetic construct
EVQLVESGGGLVQPGGSLRLSCAASGFTFNSYTMSWVRQAPGKGLEWVVTISSGGGRTYYPDSVKGRFTLSVDRSKNTLYLQMNSLRAEDTAVYYCIRGDYRYDGFAYWGQGTLVTVSS

SEQ ID NO: 13 - protein, 119 aa, synthetic construct
QVQLVQSGVEVKKPGASVKVSCAASGFTFNSYTMSWVRQAPGQGLEWMVTISSGGGRTYYPDSVKGRVTLTTDSSTTTAYMELKSLQFDDTAVYYCIRGDYRYDGFAYWGQGTLVTVSS

SEQ ID NO: 14 - protein, 107 aa, synthetic construct
DIQMTQSPSSLSASVGDRVTITCRASENIDSYLAWYQQKPGKSPQLLVYASTLLQDGVPSRFSGSGSGTDFTLTISSLQPEDVATYYCQHYYSIPYTFGSGTKLEIK

SEQ ID NO: 15 - protein, 107 aa, synthetic construct
DIQMTQSPSSLSASVGDRVTITCRASENIDSYVAWYQQKPGKAPKLLIYASTLLVTGVPSRFSGSGSGTDFTLTISSLQPEDFATYYCQHYYSIPYTFGQGTKVEIK

SEQ ID NO: 16 - protein, 107 aa, synthetic construct
EIVLTQSPATLSLSPGERATLSCRASENIDSYVAWYQQKPGQAPRLLIYASTLLVSGVPARFSGSGSGTDFTLTISSLEPEDFAVYYCQHYYSIPYTFGQGTKVEIK

SEQ ID NO: 17 - protein, 119 aa, synthetic construct
EVKLVESGGGLVKPGGSLRLSCAASGFTFNSYTMSWVRQAPGKRLEWVVTISSGGGRTYYPDSVKGRFTISRDNAKNTLYLQMSSLRAEDTAVYYCIRGDYRYDGFAYWGQGTLVTVSS

SEQ ID NO: 18 - protein, 119 aa, synthetic construct
EVKLVESGGGLVKPGGSLRLSCAASGFTFNSYTMSWVRQTPAKRLEWVVTISSGGGRTYYPDSVKGRFTISRDNAKNTLYLQMSSLRAEDTAVYYCIRGDYRYDGFAYWGQGTLVTVSS

SEQ ID NO: 19 - protein, 119 aa, synthetic construct
EVKLVESGGGLVQPGGSLRLSCAASGFTFNSYTMSWVRQAPGKRLEWVVTISSGGGRTYYPDSVKGRFTISRDNAKNTLYLQMSSLRAEDTAVYYCIRGDYRYDGFAYWGQGTLVTVSS

SEQ ID NO: 20 - protein, 119 aa, synthetic construct
EVKLVESGGGLVQPGGSLRLSCAASGFTFNSYTMSWVRQTPAKRLEWVVTISSGGGRTYYPDSVKGRFTISRDNAKNTLYLQMSSLRAEDTAVYYCIRGDYRYDGFAYWGQGTLVTVSS

SEQ ID NO: 21 - protein, 119 aa, synthetic construct
EVKLVESGGGLVKPGGSLRLSCAASGFTFNSYTMSWVRQTPAKRLEWVVTISSGGGRTYYPDSVKGRFTISRDNARNTLYLQMSSLRAEDTAVYYCIRGDYRYDGFAYWGQGTLVTVSS

SEQ ID NO: 22 - protein, 119 aa, synthetic construct
EVKLVESGGGLVKPGGSLRLSCAASGFTFNDYTMSWVRQAPGKRLEWVVTISSGGGRTYYPDSVKGRFTISRDNAKNSLYLQMNSLRAEDTAVYYCIRGDYRYDAFAYWGQGTLVTVSS

SEQ ID NO: 23 - protein, 119 aa, synthetic construct
EVQLVESGGGLVKPGGSLRLSCAASGFTFNDYTMSWVRQAPGKRLEWVVTISSGGGRTYYPDSVKGRFTISRDNAKNTLYLQMSSLRAEDTAVYYCIRGDYRYDAFAYWGQGTLVTVSS

SEQ ID NO: 24 - protein, 119 aa, synthetic construct
EVQLVESGGGLVKPGGSLRLSCAASGFTFNDYTMSWVRQAPGKRLEWVVTISSGGGRTYYPDSVKGRFTISRDNAKNSLYLQMNSLRAEDTAVYYCIRGDYRYDAFAYWGQGTLVTVSS

SEQ ID NO: 25 - protein, 107 aa, synthetic construct
DIQMTQSPSSLSASVGDRVTITCRASENIDSYLAWYQQKPGKSPQLLVYASTLLQDGVPSRFSGSRSGTDFTLTISSLQPEDVATYYCQHYYSIPYTFGSGTKLEIK

SEQ ID NO: 26 - protein, 107 aa, synthetic construct
DIQMTQSPSSLSASVGDRVTITCRASENIDSYLAWYQQKPGKSPQLLVYASTLLQDGVPSRFSGSRSGTQFTLTISSLQPEDVARYYCQHYYSIPYTFGSGTKLEIK

SEQ ID NO: 27 - protein, 107 aa, synthetic construct
DIQMTQSPSSLSASVGDRVTITCRASENIDSYLAWYQQKPGKSPQLLVYASTLLQDGVPSRFSGSRSGTQFTLTISSLQPEDFATYYCQHYYSIPYTFGSGTKLEIK

SEQ ID NO: 28 - protein, 107 aa, synthetic construct
DIQMTQSPSSLSASVGDRVTITCRASENIDSYLAWYQQKPGKSPQLLVYASTLLVDGVPSRFSGSRSGTQFSLTISSLQPEDVARYYCQHYYSIPYTFGSGTKLEIK

SEQ ID NO: 29 - protein, 119 aa, synthetic construct
EVKLVESGGGLVKPGGSLKLSCAASGFTFNEYTMSWVRQTPAKRLEWVVTISSGGGRTYYPDSVKGRFTISRDNARNTLYLQMSSLRSEDTAMYYCIRGDYRYDGFAYWGQGTLVTVST

SEQ ID NO: 30 - protein, 119 aa, synthetic construct
EVKLVESGGGLVKPGGSLKLSCAASGFTFNDYTMSWVRQTPAKRLEWVVTISSGGGRTYYPDSVKGRFTISRDNARNTLYLQMSSLRSEDTAMYYCIRGDYRYDGFAYWGQGTLVTVST

SEQ ID NO: 31 - protein, 119 aa, synthetic construct
EVKLVESGGGLVKPGGSLKLSCAASGFTFNMYTMSWVRQTPAKRLEWVVTISSGGGRTYYPDSVKGRFTISRDNARNTLYLQMSSLRSEDTAMYYCIRGDYRYDGFAYWGQGTLVTVST

SEQ ID NO: 32 - protein, 119 aa, synthetic construct
EVKLVESGGGLVKPGGSLKLSCAASGFTFNYYTMSWVRQTPAKRLEWVVTISSGGGRTYYPDSVKGRFTISRDNARNTLYLQMSSLRSEDTAMYYCIRGDYRYDGFAYWGQGTLVTVST

SEQ ID NO: 33 - protein, 119 aa, synthetic construct
EVKLVESGGGLVKPGGSLKLSCAASGFTFNPYTMSWVRQTPAKRLEWVVTISSGGGRTYYPDSVKGRFTISRDNARNTLYLQMSSLRSEDTAMYYCIRGDYRYDGFAYWGQGTLVTVST

SEQ ID NO: 34 - protein, 119 aa, synthetic construct
EVKLVESGGGLVKPGGSLKLSCAASGFTFNQYTMSWVRQTPAKRLEWVVTISSGGGRTYYPDSVKGRFTISRDNARNTLYLQMSSLRSEDTAMYYCIRGDYRYDGFAYWGQGTLVTVST

SEQ ID NO: 35 - protein, 119 aa, synthetic construct
EVKLVESGGGLVKPGGSLKLSCAASGFTFNNYTMSWVRQTPAKRLEWVVTISSGGGRTYYPDSVKGRFTISRDNARNTLYLQMSSLRSEDTAMYYCIRGDYRYDGFAYWGQGTLVTVST

SEQ ID NO: 36 - protein, 119 aa, synthetic construct
EVKLVESGGGLVKPGGSLKLSCAASGFTFNWYTMSWVRQTPAKRLEWVVTISSGGGRTYYPDSVKGRFTISRDNARNTLYLQMSSLRSEDTAMYYCIRGDYRYDGFAYWGQGTLVTVST

SEQ ID NO: 37 - protein, 119 aa, synthetic construct
EVKLVESGGGLVKPGGSLKLSCAASGFTFNAYTMSWVRQTPAKRLEWVVTISSGGGRTYYPDSVKGRFTISRDNARNTLYLQMSSLRSEDTAMYYCIRGDYRYDGFAYWGQGTLVTVST

SEQ ID NO: 38 - protein, 119 aa, synthetic construct
EVKLVESGGGLVKPGGSLKLSCAASGFTFNVYTMSWVRQTPAKRLEWVVTISSGGGRTYYPDSVKGRFTISRDNARNTLYLQMSSLRSEDTAMYYCIRGDYRYDGFAYWGQGTLVTVST

SEQ ID NO: 39 - protein, 119 aa, synthetic construct
EVKLVESGGGLVKPGGSLKLSCAASGFTFNHYTMSWVRQTPAKRLEWVVTISSGGGRTYYPDSVKGRFTISRDNARNTLYLQMSSLRSEDTAMYYCIRGDYRYDGFAYWGQGTLVTVST

SEQ ID NO: 40 - protein, 119 aa, synthetic construct
EVKLVESGGGLVKPGGSLKLSCAASGFTFNIYTMSWVRQTPAKRLEWVVTISSGGGRTYYPDSVKGRFTISRDNARNTLYLQMSSLRSEDTAMYYCIRGDYRYDGFAYWGQGTLVTVST

SEQ ID NO: 41 - protein, 119 aa, synthetic construct
EVKLVESGGGLVKPGGSLKLSCAASGFTFNRYTMSWVRQTPAKRLEWVVTISSGGGRTYYPDSVKGRFTISRDNARNTLYLQMSSLRSEDTAMYYCIRGDYRYDGFAYWGQGTLVTVST

SEQ ID NO: 42 - protein, 119 aa, synthetic construct
EVKLVESGGGLVKPGGSLKLSCAASGFTFNKYTMSWVRQTPAKRLEWVVTISSGGGRTYYPDSVKGRFTISRDNARNTLYLQMSSLRSEDTAMYYCIRGDYRYDGFAYWGQGTLVTVST

SEQ ID NO: 43 - protein, 119 aa, synthetic construct
EVKLVESGGGLVKPGGSLKLSCAASGFTFNFYTMSWVRQTPAKRLEWVVTISSGGGRTYYPDSVKGRFTISRDNARNTLYLQMSSLRSEDTAMYYCIRGDYRYDGFAYWGQGTLVTVST

SEQ ID NO: 44 - protein, 119 aa, synthetic construct
EVKLVESGGGLVKPGGSLKLSCAASGFTFNLYTMSWVRQTPAKRLEWVVTISSGGGRTYYPDSVKGRFTISRDNARNTLYLQMSSLRSEDTAMYYCIRGDYRYDGFAYWGQGTLVTVST

SEQ ID NO: 45 - protein, 119 aa, synthetic construct
EVKLVESGGGLVKPGGSLKLSCAASGFTFNSYTMSWVRQTPAKRLEWVVTISSGGGRTYYPDSVKGRFTISRDNARNTLYLQMSSLRSEDTAMYYCIRGDYRYDKFAYWGQGTLVTVST

SEQ ID NO: 46 - protein, 119 aa, synthetic construct
EVKLVESGGGLVKPGGSLKLSCAASGFTFNSYTMSWVRQTPAKRLEWVVTISSGGGRTYYPDSVKGRFTISRDNARNTLYLQMSSLRSEDTAMYYCIRGDYRYDLFAYWGQGTLVTVST

SEQ ID NO: 47 - protein, 119 aa, synthetic construct
EVKLVESGGGLVKPGGSLKLSCAASGFTFNSYTMSWVRQTPAKRLEWVVTISSGGGRTYYPDSVKGRFTISRDNARNTLYLQMSSLRSEDTAMYYCIRGDYRYDFFAYWGQGTLVTVST

SEQ ID NO: 48 - protein, 119 aa, synthetic construct
EVKLVESGGGLVKPGGSLKLSCAASGFTFNSYTMSWVRQTPAKRLEWVVTISSGGGRTYYPDSVKGRFTISRDNARNTLYLQMSSLRSEDTAMYYCIRGDYRYDRFAYWGQGTLVTVST

SEQ ID NO: 49 - protein, 119 aa, synthetic construct
EVKLVESGGGLVKPGGSLKLSCAASGFTFNSYTMSWVRQTPAKRLEWVVTISSGGGRTYYPDSVKGRFTISRDNARNTLYLQMSSLRSEDTAMYYCIRGDYRYDWFAYWGQGTLVTVST

SEQ ID NO: 50 - protein, 119 aa, synthetic construct
EVKLVESGGGLVKPGGSLKLSCAASGFTFNSYTMSWVRQTPAKRLEWVVTISSGGGRTYYPDSVKGRFTISRDNARNTLYLQMSSLRSEDTAMYYCIRGDYRYDIFAYWGQGTLVTVST

SEQ ID NO: 51 - protein, 119 aa, synthetic construct
EVKLVESGGGLVKPGGSLKLSCAASGFTFNSYTMSWVRQTPAKRLEWVVTISSGGGRTYYPDSVKGRFTISRDNARNTLYLQMSSLRSEDTAMYYCIRGDYRYDAFAYWGQGTLVTVST

SEQ ID NO: 52 - protein, 119 aa, synthetic construct
EVKLVESGGGLVKPGGSLKLSCAASGFTFNSYTMSWVRQTPAKRLEWVVTISSGGGRTYYPDSVKGRFTISRDNARNTLYLQMSSLRSEDTAMYYCIRGDYRYDYFAYWGQGTLVTVST

SEQ ID NO: 53 - protein, 119 aa, synthetic construct
EVKLVESGGGLVKPGGSLKLSCAASGFTFNSYTMSWVRQTPAKRLEWVVTISSGGGRTYYPDSVKGRFTISRDNARNTLYLQMSSLRSEDTAMYYCIRGDYRYDEFAYWGQGTLVTVST

SEQ ID NO: 54 - protein, 119 aa, synthetic construct
EVKLVESGGGLVKPGGSLKLSCAASGFTFNSYTMSWVRQTPAKRLEWVVTISSGGGRTYYPDSVKGRFTISRDNARNTLYLQMSSLRSEDTAMYYCIRGDYRYDVFAYWGQGTLVTVST

SEQ ID NO: 55 - protein, 119 aa, synthetic construct
EVKLVESGGGLVKPGGSLKLSCAASGFTFNSYTMSWVRQTPAKRLEWVVTISSGGGRTYYPDSVKGRFTISRDNARNTLYLQMSSLRSEDTAMYYCIRGDYRYDMFAYWGQGTLVTVST

SEQ ID NO: 56 - protein, 119 aa, synthetic construct
EVKLVESGGGLVKPGGSLKLSCAASGFTFNSYTMSWVRQTPAKRLEWVVTISSGGGRTYYPDSVKGRFTISRDNARNTLYLQMSSLRSEDTAMYYCIRGDYRYDNFAYWGQGTLVTVST

SEQ ID NO: 57 - protein, 119 aa, synthetic construct
EVKLVESGGGLVKPGGSLKLSCAASGFTFNSYTMSWVRQTPAKRLEWVVTISSGGGRTYYPDSVKGRFTISRDNARNTLYLQMSSLRSEDTAMYYCIRGDYRYDPFAYWGQGTLVTVST

SEQ ID NO: 58 - protein, 119 aa, synthetic construct
EVKLVESGGGLVKPGGSLKLSCAASGFTFNSYTMSWVRQTPAKRLEWVVTISSGGGRTYYPDSVKGRFTISRDNARNTLYLQMSSLRSEDTAMYYCIRGDYRYDQFAYWGQGTLVTVST

SEQ ID NO: 59 - protein, 119 aa, synthetic construct
EVKLVESGGGLVKPGGSLRLSCAASGFTFNYYTMSWVRQTPAKRLEWVVTISSGGGRTYYPDSVKGRFTISRDNAKNTLYLQMSSLRAEDTAVYYCIRGDYRYDGFAYWGQGTLVTVSS

SEQ ID NO: 60 - protein, 119 aa, synthetic construct
EVKLVESGGGLVKPGGSLRLSCAASGFTFNMYTMSWVRQTPAKRLEWVVTISSGGGRTYYPDSVKGRFTISRDNAKNTLYLQMSSLRAEDTAVYYCIRGDYRYDGFAYWGQGTLVTVSS

SEQ ID NO: 61 - protein, 119 aa, synthetic construct
EVKLVESGGGLVKPGGSLRLSCAASGFTFNQYTMSWVRQTPAKRLEWVVTISSGGGRTYYPDSVKGRFTISRDNAKNTLYLQMSSLRAEDTAVYYCIRGDYRYDGFAYWGQGTLVTVSS

SEQ ID NO: 62 - protein, 119 aa, synthetic construct
EVKLVESGGGLVKPGGSLRLSCAASGFTFNDYTMSWVRQTPAKRLEWVVTISSGGGRTYYPDSVKGRFTISRDNAKNTLYLQMSSLRAEDTAVYYCIRGDYRYDGFAYWGQGTLVTVSS

SEQ ID NO: 63 - protein, 119 aa, synthetic construct
EVKLVESGGGLVKPGGSLRLSCAASGFTFNEYTMSWVRQTPAKRLEWVVTISSGGGRTYYPDSVKGRFTISRDNAKNTLYLQMSSLRAEDTAVYYCIRGDYRYDGFAYWGQGTLVTVSS

SEQ ID NO: 64 - protein, 119 aa, synthetic construct
EVKLVESGGGLVKPGGSLRLSCAASGFTFNSYTMSWVRQTPAKRLEWVVTISSGGGRTYYPDSVKGRFTISRDNAKNTLYLQMSSLRAEDTAVYYCIRGDYRYDLFAYWGQGTLVTVSS

SEQ ID NO: 65 - protein, 119 aa, synthetic construct
EVKLVESGGGLVKPGGSLRLSCAASGFTFNSYTMSWVRQTPAKRLEWVVTISSGGGRTYYPDSVKGRFTISRDNAKNTLYLQMSSLRAEDTAVYYCIRGDYRYDIFAYWGQGTLVTVSS

SEQ ID NO: 66 - protein, 119 aa, synthetic construct
EVKLVESGGGLVKPGGSLRLSCAASGFTFNSYTMSWVRQTPAKRLEWVVTISSGGGRTYYPDSVKGRFTISRDNAKNTLYLQMSSLRAEDTAVYYCIRGDYRYDAFAYWGQGTLVTVSS

SEQ ID NO: 67 - protein, 119 aa, synthetic construct
EVKLVESGGGLVKPGGSLRLSCAASGFTFNDYTMSWVRQTPAKRLEWVVTISSGGGRTYYPDSVKGRFTISRDNAKNTLYLQMSSLRAEDTAVYYCIRGDYRYDAFAYWGQGTLVTVSS

SEQ ID NO: 68 - protein, 119 aa, synthetic construct
EVKLVESGGGLVKPGGSLRLSCAASGFTFNDYTMSWVRQTPAKGLEWVVTISSGGGRTYYPDSVKGRFTISRDNAKNTLYLQMSSLRAEDTAVYYCIRGDYRYDAFAYWGQGTLVTVSS

SEQ ID NO: 69 - protein, 107 aa, synthetic construct
DIQMTQSPSSLSASVGDRVTITCRASENIDSYLAWYQQKPGKSPQLLVYASTLLQDGVPSRFSGSRSGTQFSLTISSLQPEDVARYYCQHYYSIPYTFGSGTKLEIK

SEQ ID NO: 70 - protein, 107 aa, synthetic construct
DIQMTQSPSSLSASVGDRVTITCRASENIDSYLAWYQQKPGKSPQLLVYASTLLVDGVPSRFSGSGSGTQFSLTISSLQPEDVARYYCQHYYSIPYTFGSGTKLEIK

SEQ ID NO: 71 - protein, 107 aa, synthetic construct
DIQMTQSPSSLSASVGDRVTITCRASENIDSYLAWYQQKPGKSPQLLVYASTLLVDGVPSRFSGSRSGTDFSLTISSLQPEDVARYYCQHYYSIPYTFGSGTKLEIK

SEQ ID NO: 72 - protein, 107 aa, synthetic construct
DIQMTQSPSSLSASVGDRVTITCRASENIDSYLAWYQQKPGKSPQLLVYASTLLVDGVPSRFSGSRSGTQFSLTISSLQPEDVATYYCQHYYSIPYTFGSGTKLEIK

SEQ ID NO: 73 - protein, 30 aa, Mus musculus
EVKLVESGGGLVKPGGSLKLSCAASGFTFN

SEQ ID NO: 74 - protein, 14 aa, Mus musculus
WVRQTPAKRLEWVV

SEQ ID NO: 75 - protein, 32 aa, Mus musculus
RFTISRDNARNTLYLQMSSLRSEDTAMYYCIR

SEQ ID NO: 76 - protein, 11 aa, Mus musculus
WGQGTLVTVST

SEQ ID NO: 77 - protein, 30 aa, synthetic construct
EVKLVESGGGLVKPGGSLRLSCAASGFTFN

SEQ ID NO: 78 - protein, 14 aa, synthetic construct
WVRQAPGKRLEWVV

SEQ ID NO: 79 - protein, 32 aa, synthetic construct
RFTISRDNAKNTLYLQMSSLRAEDTAVYYCIR

SEQ ID NO: 80 - protein, 11 aa, synthetic construct
WGQGTLVTVSS

SEQ ID NO: 81 - protein, 30 aa, synthetic construct; identical to SEQ ID NO: 77

SEQ ID NO: 82 - protein, 14 aa, synthetic construct
WVRQTPAKRLEWVV

SEQ ID NO: 83 - protein, 32 aa, synthetic construct; identical to SEQ ID NO: 79

SEQ ID NO: 84 - protein, 11 aa, synthetic construct
WGQGTLVTVSS

SEQ ID NO: 85 - protein, 30 aa, synthetic construct
EVKLVESGGGLVQPGGSLRLSCAASGFTFN

SEQ ID NO: 86 - protein, 14 aa, synthetic construct
WVRQAPGKRLEWVV

SEQ ID NO: 87 - protein, 32 aa, synthetic construct; identical to SEQ ID NO: 79

SEQ ID NO: 88 - protein, 11 aa, synthetic construct
WGQGTLVTVSS

SEQ ID NO: 89 - protein, 30 aa, synthetic construct; identical to SEQ ID NO: 85

SEQ ID NO: 90 - protein, 14 aa, synthetic construct
WVRQTPAKRLEWVV

SEQ ID NO: 91 - protein, 32 aa, synthetic construct; identical to SEQ ID NO: 79

SEQ ID NO: 92 - protein, 11 aa, synthetic construct
WGQGTLVTVSS

SEQ ID NO: 93 - protein, 30 aa, synthetic construct; identical to SEQ ID NO: 77

SEQ ID NO: 94 - protein, 14 aa, synthetic construct
WVRQTPAKRLEWVV

SEQ ID NO: 95 - protein, 32 aa, synthetic construct
RFTISRDNARNTLYLQMSSLRAEDTAVYYCIR

SEQ ID NO: 96 - protein, 11 aa, synthetic construct
WGQGTLVTVSS

SEQ ID NO: 97 - protein, 30 aa, synthetic construct; identical to SEQ ID NO: 77

SEQ ID NO: 98 - protein, 14 aa, synthetic construct
WVRQAPGKRLEWVV

SEQ ID NO: 99 - protein, 32 aa, synthetic construct
RFTISRDNAKNSLYLQMNSLRAEDTAVYYCIR

SEQ ID NO: 100 - protein, 11 aa, synthetic construct
WGQGTLVTVSS

SEQ ID NO: 101 - protein, 30 aa, synthetic construct
EVQLVESGGGLVKPGGSLRLSCAASGFTFN

SEQ ID NO: 102 - protein, 14 aa, synthetic construct
WVRQAPGKRLEWVV

SEQ ID NO: 103 - protein, 32 aa, synthetic construct; identical to SEQ ID NO: 79

SEQ ID NO: 104 - protein, 11 aa, synthetic construct
WGQGTLVTVSS

SEQ ID NO: 105 - protein, 30 aa, synthetic construct; identical to SEQ ID NO: 101

SEQ ID NO: 106 - protein, 14 aa, synthetic construct
WVRQAPGKRLEWVV

SEQ ID NO: 107 - protein, 32 aa, synthetic construct; identical to SEQ ID NO: 99

SEQ ID NO: 108 - protein, 11 aa, synthetic construct
WGQGTLVTVSS

SEQ ID NO: 109 - protein, 23 aa, Mus musculus
DIQMTQSPASLSASVGETVTITC

SEQ ID NO: 110 - protein, 15 aa, Mus musculus
WYQQKQGKSPQLLVY

SEQ ID NO: 111 - protein, 32 aa, Mus musculus
GVPSRFSGSRSGTQFSLKINSLQSEDVARYYC

SEQ ID NO: 112 - protein, 10 aa, Mus musculus
FGSGTKLEIK

SEQ ID NO: 113 - protein, 23 aa, synthetic construct
DIQMTQSPSSLSASVGDRVTITC

SEQ ID NO: 114 - protein, 15 aa, synthetic construct
WYQQKPGKSPQLLVY

SEQ ID NO: 115 - protein, 32 aa, synthetic construct
GVPSRFSGSRSGTDFTLTISSLQPEDVATYYC

SEQ ID NO: 116 - protein, 10 aa, synthetic construct
FGSGTKLEIK

SEQ ID NO: 117 - protein, 23 aa, synthetic construct
DIQMTQSPSSLSASVGDRVTITC

SEQ ID NO: 118 - protein, 15 aa, synthetic construct
WYQQKPGKSPQLLVY

SEQ ID NO: 119 - protein, 32 aa, synthetic construct
GVPSRFSGSRSGTQFTLTISSLQPEDVARYYC

SEQ ID NO: 120 - protein, 10 aa, synthetic construct
FGSGTKLEIK

SEQ ID NO: 121 - protein, 23 aa, synthetic construct
DIQMTQSPSSLSASVGDRVTITC

SEQ ID NO: 122 - protein, 15 aa, synthetic construct
WYQQKPGKSPQLLVY

SEQ ID NO: 123 - protein, 32 aa, synthetic construct
GVPSRFSGSRSGTQFTLTISSLQPEDFATYYC

SEQ ID NO: 124 - protein, 10 aa, synthetic construct
FGSGTKLEIK

SEQ ID NO: 125 - protein, 23 aa, synthetic construct
DIQMTQSPSSLSASVGDRVTITC

SEQ ID NO: 126 - protein, 15 aa, synthetic construct
WYQQKPGKSPQLLVY

SEQ ID NO: 127 - protein, 32 aa, synthetic construct
GVPSRFSGSRSGTQFSLTISSLQPEDVARYYC

SEQ ID NO: 128 - protein, 10 aa, synthetic construct
FGSGTKLEIK

SEQ ID NO: 129 - protein, 23 aa, synthetic construct
DIQMTQSPSSLSASVGDRVTITC

SEQ ID NO: 130 - protein, 15 aa, synthetic construct
WYQQKPGKSPQLLVY

SEQ ID NO: 131 - protein, 31 aa, synthetic construct
VPSRFSGSRSGTDFTLTISSLQPEDVATYYC

SEQ ID NO: 132 - protein, 10 aa, synthetic construct
FGSGTKLEIK

SEQ ID NO: 133 - protein, 119 aa, synthetic construct
EVQLVESGGGLVKPGGSLRLSCAASGFTFQDYTMSWVRQAPGKRLEWVVTISSGGGRTYYPDSVKGRFTISRDNAKNSLYLQMNSLRAEDTAVYYCIRGDYRYDAFAYWGQGTLVTVSS

SEQ ID NO: 134 - protein, 119 aa, synthetic construct
EVQLVESGGGLVKPGGSLRLSCAASGFTFEDYTMSWVRQAPGKRLEWVVTISSGGGRTYYPDSVKGRFTISRDNAKNSLYLQMNSLRAEDTAVYYCIRGDYRYDAFAYWGQGTLVTVSS

SEQ ID NO: 135 - protein, 119 aa, synthetic construct
EVQLVESGGGLVKPGGSLRLSCAASGFTFHDYTMSWVRQAPGKRLEWVVTISSGGGRTYYPDSVKGRFTISRDNAKNSLYLQMNSLRAEDTAVYYCIRGDYRYDAFAYWGQGTLVTVSS

SEQ ID NO: 136 - protein, 119 aa, synthetic construct
EVQLVESGGGLVKPGGSLRLSCAASGFTFYDYTMSWVRQAPGKRLEWVVTISSGGGRTYYPDSVKGRFTISRDNAKNSLYLQMNSLRAEDTAVYYCIRGDYRYDAFAYWGQGTLVTVSS

SEQ ID NO: 137 - protein, 119 aa, synthetic construct
EVQLVESGGGLVKPGGSLRLSCAASGFTFKDYTMSWVRQAPGKRLEWVVTISSGGGRTYYPDSVKGRFTISRDNAKNSLYLQMNSLRAEDTAVYYCIRGDYRYDAFAYWGQGTLVTVSS

SEQ ID NO: 138 - protein, 119 aa, synthetic construct
EVQLVESGGGLVKPGGSLRLSCAASGFTFNDYTMSWVRQAPGKRLEWVVTISSGGGRTYYPDSVKGRFTISRDQAKNSLYLQMNSLRAEDTAVYYCIRGDYRYDAFAYWGQGTLVTVSS

SEQ ID NO: 139 - protein, 119 aa, synthetic construct
EVQLVESGGGLVKPGGSLRLSCAASGFTFNDYTMSWVRQAPGKRLEWVVTISSGGGRTYYPDSVKGRFTISRDEAKNSLYLQMNSLRAEDTAVYYCIRGDYRYDAFAYWGQGTLVTVSS

SEQ ID NO: 140 - protein, 119 aa, synthetic construct
EVQLVESGGGLVKPGGSLRLSCAASGFTFNDYTMSWVRQAPGKRLEWVVTISSGGGRTYYPDSVKGRFTISRDHAKNSLYLQMNSLRAEDTAVYYCIRGDYRYDAFAYWGQGTLVTVSS

SEQ ID NO: 141 - protein, 119 aa, synthetic construct
EVQLVESGGGLVKPGGSLRLSCAASGFTFNDYTMSWVRQAPGKRLEWVVTISSGGGRTYYPDSVKGRFTISRDYAKNSLYLQMNSLRAEDTAVYYCIRGDYRYDAFAYWGQGTLVTVSS

SEQ ID NO: 142 - protein, 119 aa, synthetic construct
EVQLVESGGGLVKPGGSLRLSCAASGFTFNDYTMSWVRQAPGKRLEWVVTISSGGGRTYYPDSVKGRFTISRDKAKNSLYLQMNSLRAEDTAVYYCIRGDYRYDAFAYWGQGTLVTVSS

SEQ ID NO: 143 - protein, 119 aa, synthetic construct
EVQLVESGGGLVKPGGSLRLSCAASGFTFQDYTMSWVRQAPGKRLEWVVTISSGGGRTYYPDSVKGRFTISRDQAKNSLYLQMNSLRAEDTAVYYCIRGDYRYDAFAYWGQGTLVTVSS

SEQ ID NO: 144 - protein, 119 aa, synthetic construct
EVQLVESGGGLVKPGGSLRLSCAASGFTFEDYTMSWVRQAPGKRLEWVVTISSGGGRTYYPDSVKGRFTISRDEAKNSLYLQMNSLRAEDTAVYYCIRGDYRYDAFAYWGQGTLVTVSS

SEQ ID NO: 145 - protein, 119 aa, synthetic construct
EVQLVESGGGLVKPGGSLRLSCAASGFTFHDYTMSWVRQAPGKRLEWVVTISSGGGRTYYPDSVKGRFTISRDHAKNSLYLQMNSLRAEDTAVYYCIRGDYRYDAFAYWGQGTLVTVSS

SEQ ID NO: 146 - protein, 119 aa, synthetic construct
EVQLVESGGGLVKPGGSLRLSCAASGFTFYDYTMSWVRQAPGKRLEWVVTISSGGGRTYYPDSVKGRFTISRDYAKNSLYLQMNSLRAEDTAVYYCIRGDYRYDAFAYWGQGTLVTVSS

SEQ ID NO: 147 - protein, 119 aa, synthetic construct
EVQLVESGGGLVKPGGSLRLSCAASGFTFKDYTMSWVRQAPGKRLEWVVTISSGGGRTYYPDSVKGRFTISRDKAKNSLYLQMNSLRAEDTAVYYCIRGDYRYDAFAYWGQGTLVTVSS

SEQ ID NO: 148 - protein, 119 aa, synthetic construct
EVQLVESGGGLVKPGGSLRLSCAASGFTFNDYTMSWVRQAPGKRLEWVVTISSGGGNTYYPDSVKGRFTISRDNAKNSLYLQMNSLRAEDTAVYYCIRGDYRYDAFAYWGQGTLVTVSS

SEQ ID NO: 149 - protein, 119 aa, synthetic construct
EVQLVESGGGLVKPGGSLRLSCAASGFTFNDYTMSWVRQAPGKRLEWVVTISSGGGQTYYPDSVKGRFTISRDNAKNSLYLQMNSLRAEDTAVYYCIRGDYRYDAFAYWGQGTLVTVSS

SEQ ID NO: 150 - protein, 119 aa, synthetic construct
EVQLVESGGGLVKPGGSLRLSCAASGFTFNDYTMSWVRQAPGKRLEWVVTISSGGGDTYYPDSVKGRFTISRDNAKNSLYLQMNSLRAEDTAVYYCIRGDYRYDAFAYWGQGTLVTVSS

SEQ ID NO: 151 - protein, 119 aa, synthetic construct
EVQLVESGGGLVKPGGSLRLSCAASGFTFNDYTMSWVRQAPGKRLEWVVTISSGGGETYYPDSVKGRFTISRDNAKNSLYLQMNSLRAEDTAVYYCIRGDYRYDAFAYWGQGTLVTVSS

SEQ ID NO: 152 - protein, 119 aa, synthetic construct
EVQLVESGGGLVKPGGSLRLSCAASGFTFNDYTMSWVRQAPGKRLEWVVTISSGGGRTYYPDSVKGRFTISRDNAKNSLYLQMNSLRAEDTAVYYCIRGDNRYDAFAYWGQGTLVTVSS

SEQ ID NO: 153 - protein, 119 aa, synthetic construct
EVQLVESGGGLVKPGGSLRLSCAASGFTFNDYTMSWVRQAPGKRLEWVVTISSGGGRTYYPDSVKGRFTISRDNAKNSLYLQMNSLRAEDTAVYYCIRGDQRYDAFAYWGQGTLVTVSS

SEQ ID NO: 154 - protein, 107 aa, synthetic construct
DIQMTQSPSSLSASVGDRVTITCRASENIDSQLAWYQQKPGKSPQLLVYASTLLVDGVPSRFSGSRSGTQFSLTISSLQPEDVARYYCQHYYSIPYTFGSGTKLEIK

SEQ ID NO: 155 - protein, 107 aa, synthetic construct
DIQMTQSPSSLSASVGDRVTITCRASENIDSRLAWYQQKPGKSPQLLVYASTLLVDGVPSRFSGSRSGTQFSLTISSLQPEDVARYYCQHYYSIPYTFGSGTKLEIK

SEQ ID NO: 156 - protein, 107 aa, synthetic construct
DIQMTQSPSSLSASVGDRVTITCRASENIDSYLAWYQQKPGKSPQLLVYASTLLVDGVPSRFSGSRSGTQFSLTISSLQPEDVARYYCQHYYSEPYTFGSGTKLEIK

SEQ ID NO: 157 - protein, 449 aa, synthetic construct
EVKLVESGGGLVKPGGSLRLSCAASGFTFNDYTMSWVRQTPAKRLEWVVTISSGGGRTYYPDSVKGRFTISRDNAKNTLYLQMSSLRAEDTAVYYCIRGDYRYDAFAYWGQGTLVTVSSASTKGPSVFPLAPSSKSTSGGTAALGCLVKDYFPEPVTVSWNSGALTSGVHTFPAVLQSSGLYSLSSVVTVPSSSLGTQTYICNVNHKPSNTKVDKKVEPKSCDKTHTCPPCPAPELLGGPSVFLFPPKPKDTLMISRTPEVTCVVVDVSHEDPEVKFNWYVDGVEVHNAKTKPREEQYNSTYRVVSVLTVLHQDWLNGKEYKCKVSNKALPAPIEKTISKAKGQPREPQVYTLPPSREEMTKNQVSLTCLVKGFYPSDIAVEWESNGQPENNYKTTPPVLDSDGSFFLYSKLTVDKSRWQQGNVFSCSVMHEALHNHYTQKSLSLSPGK

SEQ ID NO: 158 - protein, 449 aa, synthetic construct
EVQLVESGGGLVKPGGSLRLSCAASGFTFNDYTMSWVRQAPGKRLEWVVTISSGGGRTYYPDSVKGRFTISRDNAKNSLYLQMNSLRAEDTAVYYCIRGDYRYDAFAYWGQGTLVTVSSCSTKGPSVFPLAPSSKSTSGGTAALGCLVKDYFPEPVTVSWNSGALTSGVHTFPAVLQSSGLYSLSSVVTVPSSSLGTQTYICNVNHKPSNTKVDKKVEPKSCDKTHTCPPCPAPEAAGGPSVFLFPPKPKDTLMISRTPEVTCVVVCVSHEDPEVKFNWYVDGVEVHNAKTKPREEQYNSTYRVVSVLTVLHQDWLNGKEYKCKVSNKALPAPIEKTISKAKGQPREPQVYTLPPSREEMTKNQVSLTCLVKGFYPSDIAVEWESNGQPENNYKTTPPVLDSDGSFFLYSKLTVDKSRWQQGNVFSCSVMHEALHNHYTQKSLSLSPGK

SEQ ID NO: 159 - protein, 449 aa, synthetic construct
EVQLVESGGGLVKPGGSLRLSCAASGFTFNDYTMSWVRQAPGKRLEWVVTISSGGGRTYYPDSVKGRFTISRDNAKNSLYLQMNSLRAEDTAVYYCIRGDYRYDAFAYWGQGTLVTVSSASTKGPSVFPLAPSSKSTSGGTAALGCLVKDYFPEPVTVSWNSGALTSGVHTFPAVLQSSGLYSLSSVVTVPSSSLGTQTYICNVNHKPSNTKVDKKVEPKSCDKTHTCPPCPAPELLGGPSVFLFPPKPKDTLMISRTPEVTCVVVDVSHEDPEVKFNWYVDGVEVHNAKTKPREEQYNSTYRVVSVLTVLHQDWLNGKEYKCKVSNKALPAPIEKTISKAKGQPREPQVYTLPPSREEMTKNQVSLTCLVKGFYPSDIAVEWESNGQPENNYKTTPPVLDSDGSFFLYSKLTVDKSRWQQGNVFSCSVMHEALHNHYTQKSLSLSPGK

SEQ ID NO: 160 - protein, 449 aa, synthetic construct
EVQLVESGGGLVKPGGSLRLSCAASGFTFNDYTMSWVRQAPGKRLEWVVTISSGGGRTYYPDSVKGRFTISRDNAKNSLYLQMNSLRAEDTAVYYCIRGDYRYDAFAYWGQGTLVTVSSASTKGPSVFPLAPSSKSTSGGTAALGCLVKDYFPEPVTVSWNSGALTSGVHTFPAVLQSSGLYSLSSVVTVPSSSLGTQTYICNVNHKPSNTKVDKKVEPKSCDKTHTCPPCPAPELLGGPCVFLFPPKPKDTLMISRTPEVTCVVVDVSHEDPEVKFNWYVDGVEVHNAKTKPREEQYNSTYRVVSVLTVLHQDWLNGKEYKCKVSNKALPAPIEKTISKAKGQPREPQVYTLPPSREEMTKNQVSLTCLVKGFYPSDIAVEWESNGQPENNYKTTPPVLDSDGSFFLYSKLTVDKSRWQQGNVFSCSVMHEALHNHYTQKSLCLSPGK

SEQ ID NO: 161 - protein, 449 aa, synthetic construct
EVQLVESGGGLVKPGGSLRLSCAASGFTFNDYTMSWVRQAPGKRLEWVVTISSGGGRTYYPDSVKGRFTISRDNAKNSLYLQMNSLRAEDTAVYYCIRGDYRYDAFAYWGQGTLVTVSSCSTKGPSVFPLAPSSKSTSGGTAALGCLVKDYFPEPVTVSWNSGALTSGVHTFPAVLQSSGLYSLSSVVTVPSSSLGTQTYICNVNHKPSNTKVDKKVEPKSCDKTHTCPPCPAPELLGGPSVFLFPPKPKDTLMISRTPEVTCVVVDVSHEDPEVKFNWYVDGVEVHNAKTKPREEQYNSTYRVVSVLTVLHQDWLNGKEYKCKVSNKALPAPIEKTISKAKGQPREPQVYTLPPSREEMTKNQVSLTCLVKGFYPSDIAVEWESNGQPENNYKTTPPVLDSDGSFFLYSKLTVDKSRWQQGNVFSCSVMHEALHNHYTQKSLSLSPGK

SEQ ID NO: 162 - protein, 449 aa, synthetic construct
EVQLVESGGGLVKPGGSLRLSCAASGFTFNDYTMSWVRQAPGKRLEWVVTISSGGGRTYYPDSVKGRFTISRDNAKNSLYLQMNSLRAEDTAVYYCIRGDYRYDAFAYWGQGTLVTVSSASTKGPSVFPLAPSSKSTSGGTAALGCLVKDYFPEPVTVSWNSGALTSGVHTFPAVLQSSGLYSLSSVVTVPSSSLGTQTYICNVNHKPSNTKVDKKVEPKSCDKTHTCPPCPAPELLGGPCVFLFPPKPKDTLMISRTPEVTCVVVDVSHEDPEVKFNWYVDGVEVHNAKTKPREEQYNSTYRVVSVLTVLHQDWLNGKEYKCKVSNKALPAPIEKTISKAKGQPREPQVYTLPPSREEMTKNQVSLTCLVKGFYPSDIAVEWESNGQPENNYKTTPPVLDSDGSFFLYSKLTVDKSRWQQGNVFSCSVMHEALHNHYTQKSLSLSPGK

SEQ ID NO: 163 - protein, 449 aa, synthetic construct
EVQLVESGGGLVKPGGSLRLSCAASGFTFNDYTMSWVRQAPGKRLEWVVTISSGGGRTYYPDSVKGRFTISRDNAKNSLYLQMNSLRAEDTAVYYCIRGDYRYDAFAYWGQGTLVTVSSASTKGPSVFPLAPSSKSTSGGTAALGCLVKDYFPEPVTVSWNSGALTSGVHTFPAVLQSSGLYSLSSVVTVPSSSLGTQTYICNVNHKPSNTKVDKKVEPKSCDKTHTCPPCPAPELLGGPSVFLFPPKPKDTLMISRTPEVTCVVVCVSHEDPEVKFNWYVDGVEVHNAKTKPREEQYNSTYRVVSVLTVLHQDWLNGKEYKCKVSNKALPAPIEKTISKAKGQPREPQVYTLPPSREEMTKNQVSLTCLVKGFYPSDIAVEWESNGQPENNYKTTPPVLDSDGSFFLYSKLTVDKSRWQQGNVFSCSVMHEALHNHYTQKSLSLSPGK

SEQ ID NO: 164 - protein, 449 aa, synthetic construct
EVQLVESGGGLVKPGGSLRLSCAASGFTFNDYTMSWVRQAPGKRLEWVVTISSGGGRTYYPDSVKGRFTISRDNAKNSLYLQMNSLRAEDTAVYYCIRGDYRYDAFAYWGQGTLVTVSSASTKGPSVFPLAPSSKSTSGGTAALGCLVKDYFPEPVTVSWNSGALTSGVHTFPAVLQSSGLYSLSSVVTVPSSSLGTQTYICNVNHKPSNTKVDKKVEPKSSDKTHTCPPCPAPELLGGPSVFLFPPKPKDTLMISRTPEVTCVVVDVSHEDPEVKFNWYVDGVEVHNAKTKPREEQYNSTYRVVSVLTVLHQDWLNGKEYKCKVSNKALPAPIEKTISKAKGQPREPQVYTLPPSREEMTKNQVSLTCLVKGFYPSDIAVEWESNGQPENNYKTTPPVLDSDGSFFLYSKLTVDKSRWQQGNVFSCSVMHEALHNHYTQKSLCLSPGK

SEQ ID NO: 165 - protein, 449 aa, synthetic construct
EVQLVESGGGLVKPGGSLRLSCAASGFTFNDYTMSWVRQAPGKRLEWVVTISSGGGRTYYPDSVKGRFTISRDNAKNSLYLQMNSLRAEDTAVYYCIRGDYRYDAFAYWGQGTLVTVSSCSTKGPSVFPLAPSSKSTSGGTAALGCLVKDYFPEPVTVSWNSGALTSGVHTFPAVLQSSGLYSLSSVVTVPSSSLGTQTYICNVNHKPSNTKVDKKVEPKSCDKTHTCPPCPAPEAAGGPCVFLFPPKPKDTLMISRTPEVTCVVVDVSHEDPEVKFNWYVDGVEVHNAKTKPREEQYNSTYRVVSVLTVLHQDWLNGKEYKCKVSNKALPAPIEKTISKAKGQPREPQVYTLPPSREEMTKNQVSLTCLVKGFYPSDIAVEWESNGQPENNYKTTPPVLDSDGSFFLYSKLTVDKSRWQQGNVFSCSVMHEALHNHYTQKSLSLSPGK

SEQ ID NO: 166 - protein, 449 aa, synthetic construct
EVQLVESGGGLVKPGGSLRLSCAASGFTFNDYTMSWVRQAPGKRLEWVVTISSGGGRTYYPDSVKGRFTISRDNAKNSLYLQMNSLRAEDTAVYYCIRGDYRYDAFAYWGQGTLVTVSSASTKGPSVFPLAPSSKSTSGGTAALGCLVKDYFPEPVTVSWNSGALTSGVHTFPAVLQSSGLYSLSSVVTVPSSSLGTQTYICNVNHKPSNTKVDKKVEPKSCDKTHTCPPCPAPELLGGPSVFLFPPKPKDTLMISRTPEVTCVVVDVSHEDPEVKFNWYVDGVEVHNAKTKPREEQYNSTYRVVSVLTVLHQDWLNGKEYKCKVSNKALPAPIEKTISKAKGQPREPQVYTLPPSREEMTKNQVSLTCLVKGFYPSDIAVEWESNGQPENNYKTTPPVLDSDGSFFLYSKLTVDKSRWQQGNVFSCSVMHEALHNHYTQKSLCLSPGK

SEQ ID NO: 167 - protein, 449 aa, synthetic construct
EVQLVESGGGLVKPGGSLRLSCAASGFTFNDYTMSWVRQAPGKRLEWVVTISSGGGRTYYPDSVKGRFTISRDNAKNSLYLQMNSLRAEDTAVYYCIRGDYRYDAFAYWGQGTLVTVSSASTKGPSVFPLAPSSKSTSGGTAALGCLVKDYFPEPVTVSWNSGALTSGVHTFPAVLQSSGLYSLSSVVTVPSSSLGTQTYICNVNHKPSNTKVDKKVEPKSSDKTHTCPPCPAPELLGGPSVFLFPPKPKDTLMISRTPEVTCVVVDVSHEDPEVKFNWYVDGVEVHNAKTKPREEQYNSTYRVVSVLTVLHQDWLNGKEYKCKVSNKALPAPIEKTISKAKGQPREPQVYTLPPSREEMTKNQVSLTCLVKGFYPSDIAVEWESNGQPENNYKTTPPVLDSDGSFFLYSKLTVDKSRWQQGNVFSCSVMHEALHNHYTQKSLSLSPGK

SEQ ID NO: 168 - protein, 214 aa, synthetic construct
DIQMTQSPSSLSASVGDRVTITCRASENIDSYLAWYQQKPGKSPQLLVYASTLLVDGVPSRFSGSRSGTQFSLTISSLQPEDVARYYCQHYYSIPYTFGSGTKLEIKRTVAAPSVFIFPPSDEQLKSGTASVVCLLNNFYPREAKVQWCVDNALQSGNSQESVTEQDSKDSTYSLSSTLTLSKADYEKHKVYACEVTHQGLSSPVTKSFNRGEC

SEQ ID NO: 169 - protein, 214 aa, synthetic construct
DIQMTQSPSSLSASVGDRVTITCRASENIDSYLAWYQQKPGKSPQLLVYASTLLVDGVPSRFSGSRSGTQFSLTISSLQPEDVARYYCQHYYSIPYTFGSGTKLEIKRTVAAPSVFIFPPSDEQLKSGTASVVCLLNNFYPREAKVQWKVDNALQSGNSQESVTEQDSKDSTYSLSSTLTLSKADYEKHKVYACEVTHQGLSSPVTKSFNRGEC

SEQ ID NO: 170 - protein, 214 aa, synthetic construct
DIQMTQSPSSLSASVGDRVTITCRASENIDSYLAWYQQKPGKSPQLLVYASTLLVDGVPSRFSGSRSGTQFSLTISSLQPEDVARYYCQHYYSIPYTFGSGTKLEIKRTVAAPSVFIFPPSDEQLKSGTASVVCLLNNFYPREAKVQWKVDNALQSGNSQESVTEQDSKDSTYSLSSTLTLSKADYEKHKVYACEVTHQGLSSPCTKSFNRGEC

SEQ ID NO: 171 - protein, 449 aa, synthetic construct
EVQLVESGGGLVKPGGSLRLSCAASGFTFNDYTMSWVRQAPGKRLEWVVTISSGGGRTYYPDSVKGRFTISRDNAKNSLYLQMNSLRAEDTAVYYCIRGDYRYDAFAYWGQGTLVTVSSASTKGPSVFPLAPSSKSTSGGTAALGCLVKDYFPEPVTVSWNSGALTSGVHTFPAVLQSSGLYSLSSVVTVPSSSLGTQTYICNVNHKPSNTKVDKKVEPKSCDKTHTCPPCPAPEAAGGPCVFLFPPKPKDTLMISRTPEVTCVVVDVSHEDPEVKFNWYVDGVEVHNAKTKPREEQYNSTYRVVSVLTVLHQDWLNGKEYKCKVSNKALPAPIEKTISKAKGQPREPQVYTLPPSREEMTKNQVSLTCLVKGFYPSDIAVEWESNGQPENNYKTTPPVLDSDGSFFLYSKLTVDKSRWQQGNVFSCSVMHEALHNHYTQKSLCLSPGK